European Patent Application EP 4 327 823 A1, published February 28, 2024. Title: anti-CLDN4-anti-CD137 bispecific antibody. Applicant: Astellas Pharma Inc. National Cancer Center. The sequence listing filed with the application follows.

SEQUENCE LISTING (55 sequences)

SEQ ID NO: 1 - DNA, 375 bp, Artificial Sequence
  3D11 VH
  CDS (1)..(375)
caggttcagttgggacagtctggccccgaagtgaagaaacctggcgcctctgtgaaggtgtcctgcaaggcttccggctactcctttatctcctacggcatctcctgggtccgacaggctcctggacaaggcttggaatggatgggctggtcctccgtgtacaacggcaacaccaactacgtgcagaaattccagggcagagtgaccatgaccaccgacacctctgcctccaccgcctacatggaactgcggtccctgagatctgatgacgccgccgtgtactactgcgccagagactcttactcctccggctggtcttactactactccggcatggatgtgtggggccagggcacaacagtgaccgtgtcctcc

SEQ ID NO: 2 - protein, 125 aa, Artificial Sequence
  Synthetic Construct
QVQLGQSGPEVKKPGASVKVSCKASGYSFISYGISWVRQAPGQGLEWMGWSSVYNGNTNYVQKFQGRVTMTTDTSASTAYMELRSLRSDDAAVYYCARDSYSSGWSYYYSGMDVWGQGTTVTVSS

SEQ ID NO: 3 - DNA, 327 bp, Artificial Sequence
  3D11 VL
  CDS (1)..(327)
gagattgtgctgacccagtctcctggcacactgtctttgagccctggcgagagagctaccctgtcctgtagagcctctcagtccgtgtcctcctcttacctggcctggtatcagcagaagcctggacaggctccccggctgttgatctacggcgcttcttctagagccacaggcatccctgaccggttctccggatctggctctggcaccgatttcaccctgaccatcaaccggctggaacccgaggatttcgccgtgtactactgccagcagtacggctcctctccttactcttttggccagggcaccaagctggaaatcaagcgg

SEQ ID NO: 4 - protein, 109 aa, Artificial Sequence
  Synthetic Construct
EIVLTQSPGTLSLSPGERATLSCRASQSVSSSYLAWYQQKPGQAPRLLIYGASSRATGIPDRFSGSGSGTDFTLTINRLEPEDFAVYYCQQYGSSPYSFGQGTKLEIKR

SEQ ID NO: 5 - DNA, 369 bp, Artificial Sequence
  hKM3900 VH
  CDS (1)..(369)
gaagtgcagctggttcagtctggcgccgaagtgaagaaacctggcgcctccgtgaagatctcctgcaaggcttctggctacaccttcaccgactactacatgaactgggtccgacaggctcctggacagggacttgagtggatgggagatgtggtgcccaacaacggcgtgcccacctacaaccagaaattcaagggcagagtgaccatcaccgccgacaagtctacctccaccgcctacatggaactgcggagcctgagatctgaggacaccgccgtgtactactgcgccagacctcactactactacgccggcagatctggcgccatggattattggggacagggcaccctggtcaccgtgtcctct

SEQ ID NO: 6 - protein, 123 aa, Artificial Sequence
  Synthetic Construct
EVQLVQSGAEVKKPGASVKISCKASGYTFTDYYMNWVRQAPGQGLEWMGDVVPNNGVPTYNQKFKGRVTITADKSTSTAYMELRSLRSEDTAVYYCARPHYYYAGRSGAMDYWGQGTLVTVSS

SEQ ID NO: 7 - DNA, 327 bp, Artificial Sequence
  hKM3900 VL
  CDS (1)..(327)
gacatccagctgacccagtctccatcctctctgtctgcctctgtgggcgacagagtgacaattacctgcaccgcctcctccaccgtgtcctctacctacctgcactggtatcagcagaagcccggcaaggctcccaagctgctgatctactccacctccaatctggcctctggcgtgccctctagattctccggatctggctctggaaccgactataccctgacaatctccagcctgcagcctgaggacttcgccacctactactgccaccagtaccacagatccccacctacctttggccagggcaccaagctggaaatcaagcgt

SEQ ID NO: 8 - protein, 109 aa, Artificial Sequence
  Synthetic Construct
DIQLTQSPSSLSASVGDRVTITCTASSTVSSTYLHWYQQKPGKAPKLLIYSTSNLASGVPSRFSGSGSGTDYTLTISSLQPEDFATYYCHQYHRSPPTFGQGTKLEIKR

SEQ ID NO: 9 - DNA, 354 bp, Artificial Sequence
  3-34 VH
  CDS (1)..(354)
caggtccagctgcagcagtctgaggctgagctggtgaggcctggggcctcagtgaagatttcctgcaaggcttttggctacaccttcacaaaccatcatataaactgggtgaagcagaggcctggacagggcctggactggattggatatattaatccttataatgattatactaccttcaaccggaagttcaaggacaaggccacattgactgtacacaaatcctccagcacagcctatatggagcttagcggcctgacatctgacgactctgcagtctattactgtgcaagaacctggggtcactggtatttcgatctctggggccgtggcaccgtggtcactgtctcctca

SEQ ID NO: 10 - protein, 118 aa, Artificial Sequence
  Synthetic Construct
QVQLQQSEAELVRPGASVKISCKAFGYTFTNHHINWVKQRPGQGLDWIGYINPYNDYTTFNRKFKDKATLTVHKSSSTAYMELSGLTSDDSAVYYCARTWGHWYFDLWGRGTVVTVSS

SEQ ID NO: 11 - DNA, 327 bp, Artificial Sequence
  3-34 VL
  CDS (1)..(327)
gaaatagtgatgacgcagtctccagccaccctgtctgtgtctccaggggaaagagccaccctctcctgtagggccagtcagagtgttagcagcaacttagcctggtaccagcagaaacctggccaggctcccaggctcctcatctatgattcatccaccagggccactggtatcccagccaggttcagtggcagtgggtctgggacagacttcactctcaccatcagcagcctgcagtctgaagattttgcagtttattactgtcagcagtataataactggcctccgtggacgttcggccaagggaccaaggtggaaatcaaacgg

SEQ ID NO: 12 - protein, 109 aa, Artificial Sequence
  Synthetic Construct
EIVMTQSPATLSVSPGERATLSCRASQSVSSNLAWYQQKPGQAPRLLIYDSSTRATGIPARFSGSGSGTDFTLTISSLQSEDFAVYYCQQYNNWPPWTFGQGTKVEIKR

SEQ ID NO: 13 - DNA, 354 bp, Artificial Sequence
  A2-32 VH
  CDS (1)..(354)
caggtgcagctgcaggaatcgggcccaggactggtgaagccttcggagaccctgtccctcacctgcactgtctctggcggctccatcagtggttattactggagctggatccggcagcccccagggaagggcctggagtggattggatatatctattacagtggattcaccaactacaacccctccctcaagagtcgagtcaccatatcagtagacacgtccaagaaccagttctccctgaaactgagctctgtgaccgctgcggacacggccgtgtattattgtacgagagatcactcccactactactacatggacgtctggggccaagggaccacggtcaccgtctcctca

SEQ ID NO: 14 - protein, 118 aa, Artificial Sequence
  Synthetic Construct
QVQLQESGPGLVKPSETLSLTCTVSGGSISGYYWSWIRQPPGKGLEWIGYIYYSGFTNYNPSLKSRVTISVDTSKNQFSLKLSSVTAADTAVYYCTRDHSHYYYMDVWGQGTTVTVSS

SEQ ID NO: 15 - DNA, 333 bp, Artificial Sequence
  A2-32 VL
  CDS (1)..(333)
cagtctgtgctgactcagccaccctcagcgtctgggacccccgggcagagggtcaccatctcttgttctggaagcagctccaacatcggaagtaatactgtaaactggtaccagcagttcccaggaacggcccccaaactcctcatctatagtaataatcagcggccctcaggggtccctgaccgattctctggctccaagtctggcacctcagcctccctggccatcagtgggctccagtctgaggatgaggctgattattactgtgcaggatgggatgacagcctgaatggtccggtattcggcggagggaccaagctgaccgtcctaggt

SEQ ID NO: 16 - protein, 111 aa, Artificial Sequence
  Synthetic Construct
QSVLTQPPSASGTPGQRVTISCSGSSSNIGSNTVNWYQQFPGTAPKLLIYSNNQRPSGVPDRFSGSKSGTSASLAISGLQSEDEADYYCAGWDDSLNGPVFGGGTKLTVLG

SEQ ID NO: 17 - DNA, 354 bp, Artificial Sequence
  A2-48 VH
  CDS (1)..(354)
caggtgcagctgcaggagtcgggcccaggactggtgaagccttcggagaccctgtccctcacctgcactgtctctggtggctccatcagtagttactactggagctggatccggcagccccccgggaagggactggaatggattgggtatatctattacagtgggtacaccaactacaacccctccctcaagagtcgagttaacatatcagtagacacgtcccagaaccagttctccctgaagctgaattctctgaccgctgcggacacggccgtttattactgtgcgagaacacactcctattactacggtatggacgtctggggccaagggaccacggtcaccgtctcctca

SEQ ID NO: 18 - protein, 118 aa, Artificial Sequence
  Synthetic Construct
QVQLQESGPGLVKPSETLSLTCTVSGGSISSYYWSWIRQPPGKGLEWIGYIYYSGYTNYNPSLKSRVNISVDTSQNQFSLKLNSLTAADTAVYYCARTHSYYYGMDVWGQGTTVTVSS

SEQ ID NO: 19 - DNA, 333 bp, Artificial Sequence
  A2-48 VL
  CDS (1)..(333)
cagtctgtgctgactcagccaccctcagcgtctgggacccccgggcagagggtcaccatctcttgttctggaagcagctccaacatcggaaataatcctgtaaactggtaccagcagttcccaggaacggcccccaaactcctcatctatagtaataatcagcggccctcaggggtccctgaccgattctctggctccaagtctggcacctcagcctccctggccatcagtgggctccagtctgaggatgaggctgattattactgtgaagcatgggatgacagcctgaatggtccggtattcggcggagggaccaagctgaccgtcctaggt

SEQ ID NO: 20 - protein, 111 aa, Artificial Sequence
  Synthetic Construct
QSVLTQPPSASGTPGQRVTISCSGSSSNIGNNPVNWYQQFPGTAPKLLIYSNNQRPSGVPDRFSGSKSGTSASLAISGLQSEDEADYYCEAWDDSLNGPVFGGGTKLTVLG

SEQ ID NO: 21 - DNA, 363 bp, Artificial Sequence
  A2-73 VH
  CDS (1)..(363)
caggtgcagctgcaggagtcgggcccaggactggtgaagccttcggagaccctgtccctcacctgcactgtctctggtggctccatcagtagttactactggacctggatccggcagcccccagggaagggactggaattggttggatatatctattacagtggttacaccagctacaacccctccctcaagagtcgagtcaccatatcaattgacacgtccaagaaccagttctccctgcagctgaactctgtgaccgctgcggacacggccgtgtatttctgtgcgcgagatgactatggtggtaacggctactacggtgtggacgtctggggccaagggaccacggtcaccgtctcctca

SEQ ID NO: 22 - protein, 121 aa, Artificial Sequence
  Synthetic Construct
QVQLQESGPGLVKPSETLSLTCTVSGGSISSYYWTWIRQPPGKGLELVGYIYYSGYTSYNPSLKSRVTISIDTSKNQFSLQLNSVTAADTAVYFCARDDYGGNGYYGVDVWGQGTTVTVSS

SEQ ID NO: 23 - DNA, 333 bp, Artificial Sequence
  A2-73 VL
  CDS (1)..(333)
cagtctgtgctgactcagccaccctcagcgtctgggacccccgggcagagggtcaccatctcttgttctggcagcagctccaacatcggaaataatcctgtaaactggtaccggcagctcccaggaacggcccccaaactcctcatctatagtaataatcagcggccctcaggggtccctgaccgattctctggctccaagtctggcacctcagcctccctggccatcagtgggctccagtctgaggatgaggctgattattactgtgcagcatgggatgacagcctgaatggttgggtgttcggcggagggaccaagctgaccgtcctaggt

SEQ ID NO: 24 - protein, 111 aa, Artificial Sequence
  Synthetic Construct
QSVLTQPPSASGTPGQRVTISCSGSSSNIGNNPVNWYRQLPGTAPKLLIYSNNQRPSGVPDRFSGSKSGTSASLAISGLQSEDEADYYCAAWDDSLNGWVFGGGTKLTVLG

SEQ ID NO: 25 - DNA, 726 bp, Artificial Sequence
  3-34-j6 scFv
  CDS (1)..(726)
gaagttcagctgttggaaagtggtggcggactggtccagcctggcgaatctctgagactgagctgcaaggccttcgggtatacctttaccaaccaccacatcaattgggttcgacaagcccctggcaagtgcctggaatgggtcggatatatcaacccctacaacgactacaccaccttcaacgacaagttcaaggaccggttcaccctgtccgtggataagtccaagagcaccgcttacctgcagatgaactccctgagagccgaggatacagctgtgtattactgtgcccggacctggggccactggtactttgatttgtggggccagggaaccctcgtgacagtctcttctggcggcggaggaagcggaggcggaggttcaggcggcggtggatctaacatccagatgacccagtctccatccagcctgtctgcctctgtgggcgacagagtgacaattacctgtcgggcctctcagtccgtgtccagcaatctggcttggtatcagcagaagcccggcaaggctcccaagctgctgatctacgactcctccaccagagctaccggcgtgccatctagattctccggctctggctctggcaccgactttaccctgacaatttccagcctgcagcctgaggacttcgccacctactactgccagcagtacaacaactggcctccttggaccttcggctgcggcaccaaactggaaatcaagcgc

SEQ ID NO: 26 - protein, 242 aa, Artificial Sequence
  Synthetic Construct
EVQLLESGGGLVQPGESLRLSCKAFGYTFTNHHINWVRQAPGKCLEWVGYINPYNDYTTFNDKFKDRFTLSVDKSKSTAYLQMNSLRAEDTAVYYCARTWGHWYFDLWGQGTLVTVSSGGGGSGGGGSGGGGSNIQMTQSPSSLSASVGDRVTITCRASQSVSSNLAWYQQKPGKAPKLLIYDSSTRATGVPSRFSGSGSGTDFTLTISSLQPEDFATYYCQQYNNWPPWTFGCGTKLEIKR

SEQ ID NO: 27 - DNA, 732 bp, Artificial Sequence
  t2-32 scFv
  CDS (1)..(732)
caggttcagttgcaagaatctggcccaggcctcgtgaagccctccgaaacactgtctctgacctgcacagtgtccggcggctctatctctggctactactggtcctggatcagacagcctcctggcaagtgcctggaatggatcggctacatctactactctggcttcaccaactacaaccccagcctgaagtccagagtgaccatcagcgtggacacctctaagaaccagttctctctgaagctgtcctccgtgaccgccgctgataccgctgtgtattactgcacccgggaccacagccactactactacatggacgtgtggggacagggaacaaccgtgacagtctcttcaggcggtggtggatcaggcggcggaggaagtggtggcggaggttctcagtctgtgctgacccaacctccttccgcttctggcacacctggccagagagtgacaatctcttgctccggctcctcctccaacatcggctctaacaccgtgaactggtatcagcagttccccggcaccgctcctaagctgctgatctactccaacaaccagcggccttccggcgtgcccgatagattctctggctctaagtccggcacctctgccagcctggctatttctggactgcagagcgaggacgaggccgactattattgtgccggctgggacgactctctgaacggccctgtttttggctgcggcaccaaactgactgtgctgggc

SEQ ID NO: 28 - protein, 244 aa, Artificial Sequence
  Synthetic Construct
QVQLQESGPGLVKPSETLSLTCTVSGGSISGYYWSWIRQPPGKCLEWIGYIYYSGFTNYNPSLKSRVTISVDTSKNQFSLKLSSVTAADTAVYYCTRDHSHYYYMDVWGQGTTVTVSSGGGGSGGGGSGGGGSQSVLTQPPSASGTPGQRVTISCSGSSSNIGSNTVNWYQQFPGTAPKLLIYSNNQRPSGVPDRFSGSKSGTSASLAISGLQSEDEADYYCAGWDDSLNGPVFGCGTKLTVLG

SEQ ID NO: 29 - DNA, 747 bp, Artificial Sequence
  tA2-32LH scFv
  CDS (1)..(747)
caatctgttctgacccaacctccttccgcctctggcacacctggccagagagtgaccatctcttgctccggctcctcctccaacatcggctctaacaccgtgaactggtatcagcagttccccggcaccgctcctaagctgctgatctactccaacaaccagcggccttccggcgtgcccgatagattctctggctctaagtccggcacctctgccagcctggctatttctggactgcagagcgaggacgaggccgactattattgtgccggctgggacgactctctgaacggccctgtttttggcggtggcaccaaactgacagtgcttggaggcggtggtggatcaggcggcggtggaagtggtggtggtggtagcggaggtggtggatctcaggtgcagctccaagagtctggacctggcctcgtgaagccttccgagacactgtctctgacctgcacagtgtccggcggctctatctctggctactactggtcctggatcagacagcctcctggcaagggactcgagtggatcggctacatctactactctggcttcaccaactacaaccccagcctgaagtcccgcgtgaccatcagcgtggacacctctaagaaccagttctctctgaagctgtcctccgtgaccgccgctgataccgctgtgtattactgcacccgggaccacagccactactactacatggacgtgtggggacagggaacaaccgtgacagtgtcctcc

SEQ ID NO: 30 - protein, 249 aa, Artificial Sequence
  Synthetic Construct
QSVLTQPPSASGTPGQRVTISCSGSSSNIGSNTVNWYQQFPGTAPKLLIYSNNQRPSGVPDRFSGSKSGTSASLAISGLQSEDEADYYCAGWDDSLNGPVFGGGTKLTVLGGGGGSGGGGSGGGGSGGGGSQVQLQESGPGLVKPSETLSLTCTVSGGSISGYYWSWIRQPPGKGLEWIGYIYYSGFTNYNPSLKSRVTISVDTSKNQFSLKLSSVTAADTAVYYCTRDHSHYYYMDVWGQGTTVTVSS

SEQ ID NO: 31 - DNA, 732 bp, Artificial Sequence
  t2-48 scFv
  CDS (1)..(732)
caggttcagttgcaagaatctggcccaggcctcgtgaagccctccgaaacactgtctctgacctgcacagtgtccggcggctccatctcttcctactactggtcctggatcagacagcctcctggcaagtgcctggaatggatcggctacatctactactccggctacaccaactacaaccccagcctgaagtccagagtgaacatctccgtggacaccagccagaaccagttctctctgaagctgaactccctgaccgccgctgataccgctgtgtattactgcgctcggacccacagctactactatggcatggacgtgtggggacaagggacaaccgtgacagtctcttcaggcggtggtggatcaggcggcggaggaagtggtggcggaggttctcagtctgtgctgacccaacctccttccgcttctggcacacctggccagagagtgaccatcagctgtagcggctcctcctccaacatcggcaacaaccccgtgaactggtatcagcagttccccggcacagcccctaagctgctgatctactccaacaaccagcggccttccggcgtgcccgatagattctctggctctaagtccggcacctctgccagcctggctatttctggactgcagagcgaggacgaggccgactactattgcgaggcttgggacgactctctgaacggccctgtgtttggctgtggcaccaaactgactgtgctgggc

SEQ ID NO: 32 - protein, 244 aa, Artificial Sequence
  Synthetic Construct
QVQLQESGPGLVKPSETLSLTCTVSGGSISSYYWSWIRQPPGKCLEWIGYIYYSGYTNYNPSLKSRVNISVDTSQNQFSLKLNSLTAADTAVYYCARTHSYYYGMDVWGQGTTVTVSSGGGGSGGGGSGGGGSQSVLTQPPSASGTPGQRVTISCSGSSSNIGNNPVNWYQQFPGTAPKLLIYSNNQRPSGVPDRFSGSKSGTSASLAISGLQSEDEADYYCEAWDDSLNGPVFGCGTKLTVLG

SEQ ID NO: 33 - DNA, 741 bp, Artificial Sequence
  tA2-73 scFv
  CDS (1)..(741)
caggttcagttgcaagaatctggcccaggcctcgtgaagccctccgaaacactgtctctgacctgcacagtgtccggcggctccatctcttcctactactggacctggatcagacagcctcctggcaagtgcttggaactcgtgggctacatctactactccggctacaccagctacaaccccagcctgaagtccagagtgaccatcagcatcgacacctctaagaaccagttcagcctgcagctcaactccgtgaccgctgctgataccgctgtgtacttctgcgccagagatgactacggcggcaacggctattatggcgtggacgtttggggacaagggacaaccgtgacagtgtctagcggaggtggtggatcaggcggcggtggaagtggtggtggtggctctcagtctgtgctgacccaacctccttctgcctctggcacacctggccagagagtgacaatctcttgctccggctcctcctccaacatcggcaacaaccccgtgaactggtacagacagctgccaggcacagcccctaagctgctgatctactccaacaaccagcggccttccggcgtgcccgatagattctctggatctaagtccggcaccagcgccagcctggctatttctggactgcagagcgaggacgaggccgactactactgtgccgcttgggacgattctctgaacggatgggtgttcggctgcggcaccaaactgactgtgctggga

SEQ ID NO: 34 - protein, 247 aa, Artificial Sequence
  Synthetic Construct
QVQLQESGPGLVKPSETLSLTCTVSGGSISSYYWTWIRQPPGKCLELVGYIYYSGYTSYNPSLKSRVTISIDTSKNQFSLQLNSVTAADTAVYFCARDDYGGNGYYGVDVWGQGTTVTVSSGGGGSGGGGSGGGGSQSVLTQPPSASGTPGQRVTISCSGSSSNIGNNPVNWYRQLPGTAPKLLIYSNNQRPSGVPDRFSGSKSGTSASLAISGLQSEDEADYYCAAWDDSLNGWVFGCGTKLTVLG

SEQ ID NO: 35 - DNA, 2115 bp, Artificial Sequence
  hKM3900_3-34-j6  HC
  CDS (1)..(2115)
gaagtgcagctggttcagtctggcgccgaagtgaagaaacctggcgcctccgtgaagatctcctgcaaggcttctggctacaccttcaccgactactacatgaactgggtccgacaggctcctggacagggacttgagtggatgggagatgtggtgcccaacaacggcgtgcccacctacaaccagaaattcaagggcagagtgaccatcaccgccgacaagtctacctccaccgcctacatggaactgcggagcctgagatctgaggacaccgccgtgtactactgcgccagacctcactactactacgccggcagatctggcgccatggattattggggacagggcaccctggtcaccgtgtcctctgctagcacaaagggcccctctgtgttccctctggctcctagctctaagtccacctctggcggaacagctgctctgggctgtctggtcaaggactacttccctgagcctgtgaccgtgtcttggaactctggcgctctgacatccggcgtgcacacatttccagctgtgctgcagtcctccggcctgtactctctgtcctctgtcgtgaccgtgccttccagctctctgggaacccagacctacatctgcaatgtgaaccacaagccttccaacaccaaggtggacaagaaggtggaacccaagtcctgcgacaagacccacacctgtcctccatgtcctgctccagaagctgctggcggaccttccgtgttcctgtttcctccaaagcctaaggacaccctgatgatctctcggacccctgaagtgacctgcgtggtggtggatgtgtctcacgaggacccagaagtgaagttcaattggtacgtggacggcgtggaagtgcacaacgccaagaccaagcctagagaggaacagtacaactccacctacagagtggtgtccgtgctgaccgtgctgcaccaggattggctgaacggcaaagagtacaagtgcaaggtgtccaacaaggccctgcctgccggcatcgaaaagaccatctccaaggccaagggccagcctagggaaccccaggtttacaccttgccaccttctcgggacgagctgaccaagaaccaggtgtccctgacctgtctcgtgaagggcttctacccctccgatatcgccgtggaatgggagtctaatggccagcctgagaacaactacaagacaacccctcctgtgctggactccgacggctcattcttcctgtactccaagctgacagtggacaagtccagatggcagcagggcaacgtgttctcctgcagcgtgatgcacgaggccctgcacaatcactacacacagaagtctctgtctctgagccccggcaaaggtggcggaggatctggcggaggcggatccgaagttcagctgttggaaagtggtggcggactggtccagcctggcgaatctctgagactgagctgcaaggccttcgggtatacctttaccaaccaccacatcaattgggttcgacaagcccctggcaagtgcctggaatgggtcggatatatcaacccctacaacgactacaccaccttcaacgacaagttcaaggaccggttcaccctgtccgtggataagtccaagagcaccgcttacctgcagatgaactccctgagagccgaggatacagctgtgtattactgtgcccggacctggggccactggtactttgatttgtggggccagggaaccctcgtgacagtctcttctggcggcggaggaagcggaggcggaggttcaggcggcggtggatctaacatccagatgacccagtctccatccagcctgtctgcctctgtgggcgacagagtgacaattacctgtcgggcctctcagtccgtgtccagcaatctggcttggtatcagcagaagcccggcaaggctcccaagctgctgatctacgactcctccaccagagctaccggcgtgccatctagattctccggctctggctctggcaccgactttaccctgacaatttccagcctgcagcctgaggacttcgccacctactactgccagcagtacaacaactggcctccttggaccttcggctgcggcaccaaactggaaatcaagcgc

SEQ ID NO: 36 - protein, 705 aa, Artificial Sequence
  Synthetic Construct
EVQLVQSGAEVKKPGASVKISCKASGYTFTDYYMNWVRQAPGQGLEWMGDVVPNNGVPTYNQKFKGRVTITADKSTSTAYMELRSLRSEDTAVYYCARPHYYYAGRSGAMDYWGQGTLVTVSSASTKGPSVFPLAPSSKSTSGGTAALGCLVKDYFPEPVTVSWNSGALTSGVHTFPAVLQSSGLYSLSSVVTVPSSSLGTQTYICNVNHKPSNTKVDKKVEPKSCDKTHTCPPCPAPEAAGGPSVFLFPPKPKDTLMISRTPEVTCVVVDVSHEDPEVKFNWYVDGVEVHNAKTKPREEQYNSTYRVVSVLTVLHQDWLNGKEYKCKVSNKALPAGIEKTISKAKGQPREPQVYTLPPSRDELTKNQVSLTCLVKGFYPSDIAVEWESNGQPENNYKTTPPVLDSDGSFFLYSKLTVDKSRWQQGNVFSCSVMHEALHNHYTQKSLSLSPGKGGGGSGGGGSEVQLLESGGGLVQPGESLRLSCKAFGYTFTNHHINWVRQAPGKCLEWVGYINPYNDYTTFNDKFKDRFTLSVDKSKSTAYLQMNSLRAEDTAVYYCARTWGHWYFDLWGQGTLVTVSSGGGGSGGGGSGGGGSNIQMTQSPSSLSASVGDRVTITCRASQSVSSNLAWYQQKPGKAPKLLIYDSSTRATGVPSRFSGSGSGTDFTLTISSLQPEDFATYYCQQYNNWPPWTFGCGTKLEIKR

SEQ ID NO: 37 - DNA, 2136 bp, Artificial Sequence
  hKM3900_tA2-32LH HC
  CDS (1)..(2136)
gaagtgcagctggttcagtctggcgccgaagtgaagaaacctggcgcctccgtgaagatctcctgcaaggcttctggctacaccttcaccgactactacatgaactgggtccgacaggctcctggacagggacttgagtggatgggagatgtggtgcccaacaacggcgtgcccacctacaaccagaaattcaagggcagagtgaccatcaccgccgacaagtctacctccaccgcctacatggaactgcggagcctgagatctgaggacaccgccgtgtactactgcgccagacctcactactactacgccggcagatctggcgccatggattattggggacagggcaccctggtcaccgtgtcctctgctagcacaaagggcccctctgtgttccctctggctcctagctctaagtccacctctggcggaacagctgctctgggctgtctggtcaaggactacttccctgagcctgtgaccgtgtcttggaactctggcgctctgacatccggcgtgcacacatttccagctgtgctgcagtcctccggcctgtactctctgtcctctgtcgtgaccgtgccttccagctctctgggaacccagacctacatctgcaatgtgaaccacaagccttccaacaccaaggtggacaagaaggtggaacccaagtcctgcgacaagacccacacctgtcctccatgtcctgctccagaagctgctggcggaccttccgtgttcctgtttcctccaaagcctaaggacaccctgatgatctctcggacccctgaagtgacctgcgtggtggtggatgtgtctcacgaggacccagaagtgaagttcaattggtacgtggacggcgtggaagtgcacaacgccaagaccaagcctagagaggaacagtacaactccacctacagagtggtgtccgtgctgaccgtgctgcaccaggattggctgaacggcaaagagtacaagtgcaaggtgtccaacaaggccctgcctgccggcatcgaaaagaccatctccaaggccaagggccagcctagggaaccccaggtttacaccttgccaccttctcgggacgagctgaccaagaaccaggtgtccctgacctgtctcgtgaagggcttctacccctccgatatcgccgtggaatgggagtctaatggccagcctgagaacaactacaagacaacccctcctgtgctggactccgacggctcattcttcctgtactccaagctgacagtggacaagtccagatggcagcagggcaacgtgttctcctgcagcgtgatgcacgaggccctgcacaatcactacacacagaagtctctgtctctgagccccggcaaaggtggcggaggatctggcggaggcggatcccaatctgttctgacccaacctccttccgcctctggcacacctggccagagagtgaccatctcttgctccggctcctcctccaacatcggctctaacaccgtgaactggtatcagcagttccccggcaccgctcctaagctgctgatctactccaacaaccagcggccttccggcgtgcccgatagattctctggctctaagtccggcacctctgccagcctggctatttctggactgcagagcgaggacgaggccgactattattgtgccggctgggacgactctctgaacggccctgtttttggcggtggcaccaaactgacagtgcttggaggcggtggtggatcaggcggcggtggaagtggtggtggtggtagcggaggtggtggatctcaggtgcagctccaagagtctggacctggcctcgtgaagccttccgagacactgtctctgacctgcacagtgtccggcggctctatctctggctactactggtcctggatcagacagcctcctggcaagggactcgagtggatcggctacatctactactctggcttcaccaactacaaccccagcctgaagtcccgcgtgaccatcagcgtggacacctctaagaaccagttctctctgaagctgtcctccgtgaccgccgctgataccgctgtgtattactgcacccgggaccacagccactactactacatggacgtgtggggacagggaacaaccgtgacagtgtcctcc

SEQ ID NO: 38 - protein, 712 aa, Artificial Sequence
  Synthetic Construct
EVQLVQSGAEVKKPGASVKISCKASGYTFTDYYMNWVRQAPGQGLEWMGDVVPNNGVPTYNQKFKGRVTITADKSTSTAYMELRSLRSEDTAVYYCARPHYYYAGRSGAMDYWGQGTLVTVSSASTKGPSVFPLAPSSKSTSGGTAALGCLVKDYFPEPVTVSWNSGALTSGVHTFPAVLQSSGLYSLSSVVTVPSSSLGTQTYICNVNHKPSNTKVDKKVEPKSCDKTHTCPPCPAPEAAGGPSVFLFPPKPKDTLMISRTPEVTCVVVDVSHEDPEVKFNWYVDGVEVHNAKTKPREEQYNSTYRVVSVLTVLHQDWLNGKEYKCKVSNKALPAGIEKTISKAKGQPREPQVYTLPPSRDELTKNQVSLTCLVKGFYPSDIAVEWESNGQPENNYKTTPPVLDSDGSFFLYSKLTVDKSRWQQGNVFSCSVMHEALHNHYTQKSLSLSPGKGGGGSGGGGSQSVLTQPPSASGTPGQRVTISCSGSSSNIGSNTVNWYQQFPGTAPKLLIYSNNQRPSGVPDRFSGSKSGTSASLAISGLQSEDEADYYCAGWDDSLNGPVFGGGTKLTVLGGGGGSGGGGSGGGGSGGGGSQVQLQESGPGLVKPSETLSLTCTVSGGSISGYYWSWIRQPPGKGLEWIGYIYYSGFTNYNPSLKSRVTISVDTSKNQFSLKLSSVTAADTAVYYCTRDHSHYYYMDVWGQGTTVTVSS

SEQ ID NO: 39 - DNA, 645 bp, Artificial Sequence
  hKM3900 LC
  CDS (1)..(645)
gacatccagctgacccagtctccatcctctctgtctgcctctgtgggcgacagagtgacaattacctgcaccgcctcctccaccgtgtcctctacctacctgcactggtatcagcagaagcccggcaaggctcccaagctgctgatctactccacctccaatctggcctctggcgtgccctctagattctccggatctggctctggaaccgactataccctgacaatctccagcctgcagcctgaggacttcgccacctactactgccaccagtaccacagatccccacctacctttggccagggcaccaagctggaaatcaagcgtacggtggccgctccttccgtgttcatcttcccaccttccgacgagcagctgaagtccggcacagcttctgtcgtgtgcctgctgaacaacttctaccctcgggaagccaaggtgcagtggaaggtggacaatgccctgcagtccggcaactcccaagagtctgtgaccgagcaggactccaaggacagcacctacagcctgtcctccacactgaccctgtccaaggccgactacgagaagcacaaggtgtacgcctgcgaagtgacccatcagggcctgtctagccctgtgaccaagtctttcaaccggggcgagtgc

SEQ ID NO: 40 - protein, 215 aa, Artificial Sequence
  Synthetic Construct
DIQLTQSPSSLSASVGDRVTITCTASSTVSSTYLHWYQQKPGKAPKLLIYSTSNLASGVPSRFSGSGSGTDYTLTISSLQPEDFATYYCHQYHRSPPTFGQGTKLEIKRTVAAPSVFIFPPSDEQLKSGTASVVCLLNNFYPREAKVQWKVDNALQSGNSQESVTEQDSKDSTYSLSSTLTLSKADYEKHKVYACEVTHQGLSSPVTKSFNRGEC

SEQ ID NO: 41 - protein, 486 aa, Artificial Sequence
  anti-CD3 scFv-human Fc fusion protein
  PEPTIDE (1)..(486)
EVQLVESGGGLIQPGGSLRLSCAASGFTFNTYAMNWVRQAPGKGLEWVARIRSKYNNYATYYADSVKDRFTISRDDSKSTLYLQMNNLRAEDTAVYYCVRHGNFGNSYVSWFAYWGQGTLVTVSSGKPGSGKPGSGKPGSGKPGSQAVVTQEPSLTVSPGGTVTLTCRSSTGAVTTSNYANWVQQKPGQAPRGLIGGTNKRAPGTPARFSGSLLGDKAALTLSGAQPEDEAEYYCALWYSNLWVFGSGTKVTVLEPKSSDKTHTCPPCPAPEAAGGPSVFLFPPKPKDTLMISRTPEVTCVVVDVSHEDPEVKFNWYVDGVEVHNAKTKPREEQYASTYRVVSVLTVLHQDWLNGKEYKCKVSNKALPAPIEKTISKAKGQPREPQVYTLPPSRDELTKNQVSLWCLVKGFYPSDIAVEWESNGQPENNYKTTPPVLDSDGSFFLYSKLTVDKSRWQQGNVFSCSVMHEALHNHYTQKSLSLSPGK

SEQ ID NO: 42 - protein, 255 aa, Homo sapiens
  PEPTIDE (1)..(255)
MGNSCYNIVATLLLVLNFERTRSLQDPCSNCPAGTFCDNNRNQICSPCPPNSFSSAGGQRTCDICRQCKGVFRTRKECSSTSNAECDCTPGFHCLGAGCSMCEQDCKQGQELTKKGCKDCCFGTFNDQKRGICRPWTNCSLDGKSVLVNGTKERDVVCGPSPADLSPGASSVTPPAPAREPGHSPQIISFFLALTSTALLFLLFFLTLRFSVVKRGRKKLLYIFKQPFMRPVQTTQEEDGCSCRFPEEEEGGCEL

SEQ ID NO: 43 - protein, 254 aa, Macaca fascicularis
  PEPTIDE (1)..(254)
MGNSCYNIVATLLLVLNFERTRSLQDLCSNCPAGTFCDNNRSQICSPCPPNSFSSAGGQRTCDICRQCKGVFKTRKECSSTSNAECDCISGYHCLGAECSMCEQDCKQGQELTKKGCKDCCFGTFNDQKRGICRPWTNCSLDGKSVLVNGTKERDVVCGPSPADLSPGASSATPPAPAREPGHSPQIIFFLALTSTVVLFLLFFLVLRFSVVKRSRKKLLYIFKQPFMRPVQTTQEEDGCSCRFPEEEEGGCEL

SEQ ID NO: 44 - protein, 6 aa, Artificial Sequence
  His tag protein
  PEPTIDE (1)..(6)
HHHHHH

SEQ ID NO: 45 - protein, 26 aa, Artificial Sequence
  3xFLAG tag protein E
  PEPTIDE (1)..(26)
DYKDDDDKGDYKDDDDKIDYKDDDDK

SEQ ID NO: 46 - protein, 4 aa, Artificial Sequence
  GS linker
  PEPTIDE (1)..(4)
GGGS

SEQ ID NO: 47 - protein, 4 aa, Artificial Sequence
  GS linker
  PEPTIDE (1)..(4)
SGGG

SEQ ID NO: 48 - protein, 5 aa, Artificial Sequence
  GS linker
  PEPTIDE (1)..(5)
GGGGS

SEQ ID NO: 49 - protein, 5 aa, Artificial Sequence
  GS linker
  PEPTIDE (1)..(5)
SGGGG

SEQ ID NO: 50 - protein, 6 aa, Artificial Sequence
  GS linker
  PEPTIDE (1)..(6)
GGGGGS

SEQ ID NO: 51 - protein, 6 aa, Artificial Sequence
  GS linker
  PEPTIDE (1)..(6)
SGGGGG

SEQ ID NO: 52 - protein, 7 aa, Artificial Sequence
  GS linker
  PEPTIDE (1)..(7)
GGGGGGS

SEQ ID NO: 53 - protein, 7 aa, Artificial Sequence
  GS linker
  PEPTIDE (1)..(7)
SGGGGGG

SEQ ID NO: 54 - protein, 10 aa, Artificial Sequence
  GS linker
  PEPTIDE (1)..(10)
GGGGSGGGGS

SEQ ID NO: 55 - protein, 5 aa, Artificial Sequence
  GKPGS linker
  PEPTIDE (1)..(5)
GKPGS